European Patent Application EP 4 130 038 A1, published February 8, 2023. Title: Anti-IL-2 antibody, complex comprising it, and uses thereof. Applicant: Institut national de recherche pour l’agriculture, l’alimentation et l’environnement Université de Nantes INSTITUT NATIONAL DE LA SANTE ET DE LA RECHERCHE MEDICALE (INSERM). The sequence listing filed with the application follows.

SEQUENCE LISTING (20 sequences)

SEQ ID NO: 1 - DNA, 21 bp, Artificial Sequence
  "nucleic acid sequence coding for H-CDR1 of the anti-human IL-2 antibody of the invention"
  nucleic acid sequence coding for H-CDR1 of the anti-human IL-2 antibody of the invention
agtagtagttattgctggcac

SEQ ID NO: 2 - DNA, 48 bp, Artificial Sequence
  "nucleic acid sequence coding for H-CDR2 of the anti-human IL-2 antibody of the invention"
  nucleic acid sequence coding for H-CDR2 of the anti-human IL-2 antibody of the invention
cgcatatgttatgaaggttcaatatactatagtccatccatcaaaagc

SEQ ID NO: 3 - DNA, 42 bp, Artificial Sequence
  "nucleic acid sequence coding for H-CDR3 of the anti-human IL-2 antibody of the invention"
  nucleic acid sequence coding for H-CDR3 of the anti-human IL-2 antibody of the invention
gaaaactggggctatggacccaacccttatgctatggactac

SEQ ID NO: 4 - DNA, 372 bp, Artificial Sequence
  "nucleic acid sequence coding for the heavy variable domain of the anti-human IL-2 antibody of the invention, without a leader sequence"
  nucleic acid sequence coding for the heavy variable domain of the anti-human IL-2 antibody of the invention, without a leader sequence
cagattcagcttaaggagtctggacctgctgtcatcaagccatcacagtcactgtctctcacctgcatagtctctggattctccatcacaagtagtagttattgctggcactggatccgccagcccccaggaaaggggttagagtggatggggcgcatatgttatgaaggttcaatatactatagtccatccatcaaaagccgcagcaccatctccagagacacatctctgaacaaattctttatccagctgagctctgtgacaaatgaggacacagccatgtactactgttccagggaaaactggggctatggacccaacccttatgctatggactactggggtcaaggaacctcagtcaccgtctcctca

SEQ ID NO: 5 - DNA, 429 bp, Artificial Sequence
  "nucleic acid sequence coding for the heavy variable domain of the anti-human IL-2 antibody of the invention, with a leader sequence"
  nucleic acid sequence coding for the heavy variable domain of the anti-human IL-2 antibody of the invention, with a leader sequence
atgagactactagggtttctcctgtgcttggcagcagctctaaaaagtgttctgtcccagattcagcttaaggagtctggacctgctgtcatcaagccatcacagtcactgtctctcacctgcatagtctctggattctccatcacaagtagtagttattgctggcactggatccgccagcccccaggaaaggggttagagtggatggggcgcatatgttatgaaggttcaatatactatagtccatccatcaaaagccgcagcaccatctccagagacacatctctgaacaaattctttatccagctgagctctgtgacaaatgaggacacagccatgtactactgttccagggaaaactggggctatggacccaacccttatgctatggactactggggtcaaggaacctcagtcaccgtctcctca

SEQ ID NO: 6 - DNA, 42 bp, Artificial Sequence
  "nucleic acid sequence coding for L-CDR1 of the anti-human IL-2 antibody of the invention"
  nucleic acid sequence coding for L-CDR1 of the anti-human IL-2 antibody of the invention
cgctcaagtactggggctgttacaactagtaactatgccaac

SEQ ID NO: 7 - DNA, 21 bp, Artificial Sequence
  "nucleic acid sequence coding for L-CDR2 of the anti-human IL-2 antibody of the invention"
  nucleic acid sequence coding for L-CDR2 of the anti-human IL-2 antibody of the invention
ggtaccagcaaccgagctcca

SEQ ID NO: 8 - DNA, 27 bp, Artificial Sequence
  "nucleic acid sequence coding for L-CDR3 of the anti-human IL-2 antibody of the invention"
  nucleic acid sequence coding for L-CDR3 of the anti-human IL-2 antibody of the invention
gctctatggtacagcacccattttgtt

SEQ ID NO: 9 - DNA, 327 bp, Artificial Sequence
  "nucleic acid sequence coding for the light variable domain of the anti-human IL-2 antibody of the invention, without a leader sequence"
  nucleic acid sequence coding for the light variable domain of the anti-human IL-2 antibody of the invention, without a leader sequence
caggctgttgtgactcaggaatctgcactcaccacatcacctggtggaacagtcatactcacttgtcgctcaagtactggggctgttacaactagtaactatgccaactgggtccaagaaaaaccagatcatttattcactggtctaataggtggtaccagcaaccgagctccaggtgttcctgtcagattctcaggctccctgattggagacaaggctgccctcaccatcacaggggcacagactgaggatgatgcaatgtatttctgtgctctatggtacagcacccattttgttttcggcggtggaaccaaggtcactgtccta

SEQ ID NO: 10 - DNA, 384 bp, Artificial Sequence
  "nucleic acid sequence coding for the light variable domain of the anti-human IL-2 antibody of the invention, with a leader sequence"
  nucleic acid sequence coding for the light variable domain of the anti-human IL-2 antibody of the invention, with a leader sequence
atggcctggacttcacttatactctctctcctggctctctgctcaggagccagttcccaggctgttgtgactcaggaatctgcactcaccacatcacctggtggaacagtcatactcacttgtcgctcaagtactggggctgttacaactagtaactatgccaactgggtccaagaaaaaccagatcatttattcactggtctaataggtggtaccagcaaccgagctccaggtgttcctgtcagattctcaggctccctgattggagacaaggctgccctcaccatcacaggggcacagactgaggatgatgcaatgtatttctgtgctctatggtacagcacccattttgttttcggcggtggaaccaaggtcactgtccta

SEQ ID NO: 11 - protein, 7 aa, Artificial Sequence
  "amino acid sequence of H-CDR1 of the anti-human IL-2 antibody of the invention"
  amino acid sequence of H-CDR1 of the anti-human IL-2 antibody of the invention
SSSYCWH

SEQ ID NO: 12 - protein, 16 aa, Artificial Sequence
  "amino acid sequence of H-CDR2 of the anti-human IL-2 antibody of the invention"
  amino acid sequence of H-CDR2 of the anti-human IL-2 antibody of the invention
RICYEGSIYYSPSIKS

SEQ ID NO: 13 - protein, 14 aa, Artificial Sequence
  "amino acid sequence of H-CDR3 of the anti-human IL-2 antibody of the invention"
  amino acid sequence of H-CDR3 of the anti-human IL-2 antibody of the invention
ENWGYGPNPYAMDY

SEQ ID NO: 14 - protein, 124 aa, Artificial Sequence
  "amino acid sequence of the heavy variable domain of the anti-human IL-2 antibody of the invention, without a leader sequence"
  amino acid sequence of the heavy variable domain of the anti-human IL-2 antibody of the invention, without a leader sequence
QIQLKESGPAVIKPSQSLSLTCIVSGFSITSSSYCWHWIRQPPGKGLEWMGRICYEGSIYYSPSIKSRSTISRDTSLNKFFIQLSSVTNEDTAMYYCSRENWGYGPNPYAMDYWGQGTSVTVSS

SEQ ID NO: 15 - protein, 143 aa, Artificial Sequence
  "amino acid sequence of the heavy variable domain of the anti-human IL-2 antibody of the invention, with a leader sequence"
  amino acid sequence of the heavy variable domain of the anti-human IL-2 antibody of the invention, with a leader sequence
MRLLGFLLCLAAALKSVLSQIQLKESGPAVIKPSQSLSLTCIVSGFSITSSSYCWHWIRQPPGKGLEWMGRICYEGSIYYSPSIKSRSTISRDTSLNKFFIQLSSVTNEDTAMYYCSRENWGYGPNPYAMDYWGQGTSVTVSS

SEQ ID NO: 16 - protein, 14 aa, Artificial Sequence
  "amino acid sequence of L-CDR1 of the anti-human IL-2 antibody of the invention"
  amino acid sequence of L-CDR1 of the anti-human IL-2 antibody of the invention
RSSTGAVTTSNYAN

SEQ ID NO: 17 - protein, 7 aa, Artificial Sequence
  "amino acid sequence of L-CDR2 of the anti-human IL-2 antibody of the invention"
  amino acid sequence of L-CDR2 of the anti-human IL-2 antibody of the invention
GTSNRAP

SEQ ID NO: 18 - protein, 9 aa, Artificial Sequence
  "amino acid sequence of L-CDR3 of the anti-human IL-2 antibody of the invention"
  amino acid sequence of L-CDR3 of the anti-human IL-2 antibody of the invention
ALWYSTHFV

SEQ ID NO: 19 - protein, 109 aa, Artificial Sequence
  "amino acid sequence of the light variable domain of the anti-human IL-2 antibody of the invention, without a leader sequence"
  amino acid sequence of the light variable domain of the anti-human IL-2 antibody of the invention, without a leader sequence
QAVVTQESALTTSPGGTVILTCRSSTGAVTTSNYANWVQEKPDHLFTGLIGGTSNRAPGVPVRFSGSLIGDKAALTITGAQTEDDAMYFCALWYSTHFVFGGGTKVTVL

SEQ ID NO: 20 - protein, 128 aa, Artificial Sequence
  "amino acid sequence of the light variable domain of the anti-human IL-2 antibody of the invention, with a leader sequence"
  amino acid sequence of the light variable domain of the anti-human IL-2 antibody of the invention, with a leader sequence
MAWTSLILSLLALCSGASSQAVVTQESALTTSPGGTVILTCRSSTGAVTTSNYANWVQEKPDHLFTGLIGGTSNRAPGVPVRFSGSLIGDKAALTITGAQTEDDAMYFCALWYSTHFVFGGGTKVTVL